European Patent Specification EP 4 168 439 B1, published July 31, 2024. Title: BINDING PROTEIN SPECIFIC FOR THE SPIKE PROTEIN OF SEVERE ACUTE RESPIRATORY SYNDROME CORONA VIRUS 2 (SARS-COV-2). Applicant: Navigo Proteins GmbH. The sequence listing filed with the application follows.

SEQUENCE LISTING (72 sequences)

SEQ ID NO: 1 - protein, 58 aa, Artificial Sequence
  spike protein binding protein 212434
NAAVLDIAQHSATEEIWWLPNLTKQQKVWFIMSLTQDPSVSKEVLGEAQKLNDSQAPK

SEQ ID NO: 2 - protein, 58 aa, Artificial Sequence
  spike protein binding protein
IAAKFDEAQQYAFYKILHLWNLTEEQRNAFIQSLRDDPSVSLEVLGEARKLNTSQAPK

SEQ ID NO: 3 - protein, 58 aa, Artificial Sequence
  spike protein binding protein
IAAKFDEAQLAAFQEIRHLPNLTEEQREAFITSLYDDPSVSLEVLGEAQKLNDSQAPK

SEQ ID NO: 4 - protein, 58 aa, Artificial Sequence
  spike protein binding protein
  misc_feature (17)..(17): Xaa can be any naturally occurring amino acid
  misc_feature (28)..(28): Xaa can be any naturally occurring amino acid
  misc_feature (32)..(32): Xaa can be any naturally occurring amino acid
  misc_feature (35)..(35): Xaa can be any naturally occurring amino acid
IAAKFDEAQYAAFLEIXHLPNLTEEQRXAFIXSLXDDPSVSLEVLGEAQKLNDSQAPK

SEQ ID NO: 5 - protein, 58 aa, Artificial Sequence
  spike protein binding protein
IAAKFDEAQYAAFLEIVHLPNLTEEQRQAFIASLWDDPSVSLEVLGEAQKLNDSQAPK

SEQ ID NO: 6 - protein, 58 aa, Artificial Sequence
  spike protein binding protein
IAAKFDEAQYAAFLEIHHLPNLTEEQRHAFILSLYDDPSVSLEVLGEAQKLNDSQAPK

SEQ ID NO: 7 - protein, 116 aa, Artificial Sequence
  spike protein binding protein 212361
IAAKFDEAQQYAFYKILHLWNLTEEQRNAFIQSLRDDPSVSLEVLGEARKLNTSQAPKIAAKFDEAQYAAFLEIVHLPNLTEEQRQAFIASLWDDPSVSLEVLGEAQKLNDSQAPK

SEQ ID NO: 8 - protein, 116 aa, Artificial Sequence
  spike protein binding protein 212335
IAAKFDEAQQYAFYKILHLWNLTEEQRNAFIQSLRDDPSVSLEVLGEARKLNTSQAPKIAAKFDEAQYAAFLEIHHLPNLTEEQRHAFILSLYDDPSVSLEVLGEAQKLNDSQAPK

SEQ ID NO: 9 - protein, 116 aa, Artificial Sequence
  spike protein binding protein 213103
IAAKFDEAQQWAFYEILHLENLTEEQRNAFIQSLRDDPSVSREVLGEATKLNTSQAPKIAAKFDEAQLAAFQEIRHLPNLTEEQREAFITSLYDDPSVSLEVLGEAQKLNDSQAPK

SEQ ID NO: 10 - protein, 1273 aa, Artificial Sequence
  spike glycoprotein S
MFVFLVLLPLVSSQCVNLTTRTQLPPAYTNSFTRGVYYPDKVFRSSVLHSTQDLFLPFFSNVTWFHAIHVSGTNGTKRFDNPVLPFNDGVYFASTEKSNIIRGWIFGTTLDSKTQSLLIVNNATNVVIKVCEFQFCNDPFLGVYYHKNNKSWMESEFRVYSSANNCTFEYVSQPFLMDLEGKQGNFKNLREFVFKNIDGYFKIYSKHTPINLVRDLPQGFSALEPLVDLPIGINITRFQTLLALHRSYLTPGDSSSGWTAGAAAYYVGYLQPRTFLLKYNENGTITDAVDCALDPLSETKCTLKSFTVEKGIYQTSNFRVQPTESIVRFPNITNLCPFGEVFNATRFASVYAWNRKRISNCVADYSVLYNSASFSTFKCYGVSPTKLNDLCFTNVYADSFVIRGDEVRQIAPGQTGKIADYNYKLPDDFTGCVIAWNSNNLDSKVGGNYNYLYRLFRKSNLKPFERDISTEIYQAGSTPCNGVEGFNCYFPLQSYGFQPTNGVGYQPYRVVVLSFELLHAPATVCGPKKSTNLVKNKCVNFNFNGLTGTGVLTESNKKFLPFQQFGRDIADTTDAVRDPQTLEILDITPCSFGGVSVITPGTNTSNQVAVLYQDVNCTEVPVAIHADQLTPTWRVYSTGSNVFQTRAGCLIGAEHVNNSYECDIPIGAGICASYQTQTNSPRRARSVASQSIIAYTMSLGAENSVAYSNNSIAIPTNFTISVTTEILPVSMTKTSVDCTMYICGDSTECSNLLLQYGSFCTQLNRALTGIAVEQDKNTQEVFAQVKQIYKTPPIKDFGGFNFSQILPDPSKPSKRSFIEDLLFNKVTLADAGFIKQYGDCLGDIAARDLICAQKFNGLTVLPPLLTDEMIAQYTSALLAGTITSGWTFGAGAALQIPFAMQMAYRFNGIGVTQNVLYENQKLIANQFNSAIGKIQDSLSSTASALGKLQDVVNQNAQALNTLVKQLSSNFGAISSVLNDILSRLDKVEAEVQIDRLITGRLQSLQTYVTQQLIRAAEIRASANLAATKMSECVLGQSKRVDFCGKGYHLMSFPQSAPHGVVFLHVTYVPAQEKNFTTAPAICHDGKAHFPREGVFVSNGTHWFVTQRNFYEPQIITTDNTFVSGNCDVVIGIVNNTVYDPLQPELDSFKEELDKYFKNHTSPDVDLGDISGINASVVNIQKEIDRLNEVAKNLNESLIDLQELGKYEQYIKWPWYIWLGFIAGLIAIVMVTIMLCCMTSCCSCLKGCCSCGSCCKFDEDDSEPVLKGVKLHYT

SEQ ID NO: 11 - protein, 670 aa, Artificial Sequence
  S1 domain of spike protein
VNLTTRTQLPPAYTNSFTRGVYYPDKVFRSSVLHSTQDLFLPFFSNVTWFHAIHVSGTNGTKRFDNPVLPFNDGVYFASTEKSNIIRGWIFGTTLDSKTQSLLIVNNATNVVIKVCEFQFCNDPFLGVYYHKNNKSWMESEFRVYSSANNCTFEYVSQPFLMDLEGKQGNFKNLREFVFKNIDGYFKIYSKHTPINLVRDLPQGFSALEPLVDLPIGINITRFQTLLALHRSYLTPGDSSSGWTAGAAAYYVGYLQPRTFLLKYNENGTITDAVDCALDPLSETKCTLKSFTVEKGIYQTSNFRVQPTESIVRFPNITNLCPFGEVFNATRFASVYAWNRKRISNCVADYSVLYNSASFSTFKCYGVSPTKLNDLCFTNVYADSFVIRGDEVRQIAPGQTGKIADYNYKLPDDFTGCVIAWNSNNLDSKVGGNYNYLYRLFRKSNLKPFERDISTEIYQAGSTPCNGVEGFNCYFPLQSYGFQPTNGVGYQPYRVVVLSFELLHAPATVCGPKKSTNLVKNKCVNFNFNGLTGTGVLTESNKKFLPFQQFGRDIADTTDAVRDPQTLEILDITPCSFGGVSVITPGTNTSNQVAVLYQDVNCTEVPVAIHADQLTPTWRVYSTGSNVFQTRAGCLIGAEHVNNSYECDIPIGAGICASYQTQTNSPRRAR

SEQ ID NO: 12 - protein, 223 aa, Artificial Sequence
  receptor binding domain (RBD) of spike protein
RVQPTESIVRFPNITNLCPFGEVFNATRFASVYAWNRKRISNCVADYSVLYNSASFSTFKCYGVSPTKLNDLCFTNVYADSFVIRGDEVRQIAPGQTGKIADYNYKLPDDFTGCVIAWNSNNLDSKVGGNYNYLYRLFRKSNLKPFERDISTEIYQAGSTPCNGVEGFNCYFPLQSYGFQPTNGVGYQPYRVVVLSFELLHAPATVCGPKKSTNLVKNKCVNF

SEQ ID NO: 13 - protein, 58 aa, Artificial Sequence
  PAdelFc
IAAQHDKDQSAADSEILHLPNLTEEQRNAFRQSLSDDPSVSLEILAEAKKLNDAQAPK

SEQ ID NO: 14 - protein, 58 aa, Artificial Sequence
  PAdelFc non-immunoglobulin binding protein
IAAQHDKIQQAADKEILHLPNLTEEQRNKFRQSLRDDPSVSAEILAEAKKLNDAQAPK

SEQ ID NO: 15 - protein, 58 aa, Artificial Sequence
  Ig binding protein cs27 as scaffold
IAAKFDEAQQAAFYEILHLPNLTEEQRNAFIQSLRDDPSVSLEVLGEAQKLNDSQAPK

SEQ ID NO: 16 - protein, 58 aa, Artificial Sequence
  Ig binding protein C27 as scaffold
NAAKFDEAQQSAFYEILHLPNLTEEQRNAFIQSLKDDPSVSKEVLGEAQKLNDSQAPK

SEQ ID NO: 17 - protein, 116 aa, Artificial Sequence
  spike protein binding protein 212860
IAAKFDEAQQYAFYKILHLWNLTEEQRNAFIQSLRDDPSVSLEVLGEARKLNTSQAPKIAAKFDEAQYAAFLEIQHLPNLTEEQRQAFIVSLADDPSVSLEVLGEAQKLNDSQAPK

SEQ ID NO: 18 - protein, 116 aa, Artificial Sequence
  spike protein binding protein 212728
IAAKFDEAQLAAFEEIRHLPNLTEEQREAFITSLYDDPSVSLEVLGEAQKLNDSQAPKIAAKFDEAQQAAFYEILHLPNPTEWQRNYFIQQLRDDPSVSLAVLGRAQVLNDSQAPK

SEQ ID NO: 19 - protein, 116 aa, Artificial Sequence
  spike protein binding protein 212522
IAAKFDEAQQAAFYEILHLPNLTELQRNWFIQLLRDDPSVSLQVLGHAQYLNDSQAPKIAAKFDEAQQYAFYQILHLHNLTEEQRNAFIQSLRDDPSVSHEVLGEAKKLNESQAPK

SEQ ID NO: 20 - protein, 58 aa, Artificial Sequence
  SPike protein binding protein
  Xaa (14)..(14)
  Xaa (14)..(14): Xaa may be any amino acid, preferably Q or E
IAAKFDEAQLAAFXEIRHLPNLTEEQREAFITSLYDDPSVSLEVLGEAQKLNDSQAPK

SEQ ID NO: 21 - protein, 58 aa, Artificial Sequence
  Spike protein binding protein
IAAKFDEAQLAAFEEIRHLPNLTEEQREAFITSLYDDPSVSLEVLGEAQKLNDSQAPK

SEQ ID NO: 22 - protein, 58 aa, Artificial Sequence
  Spike protein binding protein
IAAKFDEAQQAAFYEILHLPNPTEWQRNYFIQQLRDDPSVSLAVLGRAQVLNDSQAPK

SEQ ID NO: 23 - protein, 58 aa, Artificial Sequence
  Spike protein binding protein
IAAKFDEAQYAAFLEIQHLPNLTEEQRQAFIVSLADDPSVSLEVLGEAQKLNDSQAPK

SEQ ID NO: 24 - protein, 58 aa, Artificial Sequence
  Spike protein binding protein
IAAKFDEAQQAAFYEILHLPNLTELQRNWFIQLLRDDPSVSLQVLGHAQYLNDSQAPK

SEQ ID NO: 25 - protein, 58 aa, Artificial Sequence
  Spike protein binding protein
IAAKFDEAQQYAFYQILHLHNLTEEQRNAFIQSLRDDPSVSHEVLGEAKKLNESQAPK

SEQ ID NO: 26 - protein, 58 aa, Artificial Sequence
  Spike protein binding protein
IAAKFDEAQQWAFYEILHLENLTEEQRNAFIQSLRDDPSVSREVLGEATKLNTSQAPK

SEQ ID NO: 27 - protein, 56 aa, Artificial Sequence
  Spike binding protein 212434 Ndel2
AVLDIAQHSATEEIWWLPNLTKQQKVWFIMSLTQDPSVSKEVLGEAQKLNDSQAPK

SEQ ID NO: 28 - protein, 56 aa, Artificial Sequence
  spike binding protein 212896
AVLDIDQHAATEEIWWLPNLTKQQKVWFIMSLTQDPSVSLEILAEAKKLNDAQAPK

SEQ ID NO: 29 - protein, 231 aa, Artificial Sequence
  fusion protein 212895 (fusion of 212434 with (PAdelFc)3)
AVLDIAQHSATEEIWWLPNLTKQQKVWFIMSLTQDPSVSKEVLGEAQKLNDSQAPKIAAQHDKIQQAADKEILHLPNLTEEQRNKFRQSLRDDPSVSAEILAEAKKLNDAQAPKIAAQHDKIQQAADKEILHLPNLTEEQRNKFRQSLRDDPSVSAEILAEAKKLNDAQAPKIAAQHDKIQQAADKEILHLPNLTEEQRNKFRQSLRDDPSVSAEILAEAKKLNDAQAPKC

SEQ ID NO: 30 - protein, 231 aa, Artificial Sequence
  fusion protein 212896 (fusion of 212896 with (PAdelFc)3)
AVLDIDQHAATEEIWWLPNLTKQQKVWFIMSLTQDPSVSLEILAEAKKLNDAQAPKIAAQHDKIQQAADKEILHLPNLTEEQRNKFRQSLRDDPSVSAEILAEAKKLNDAQAPKIAAQHDKIQQAADKEILHLPNLTEEQRNKFRQSLRDDPSVSAEILAEAKKLNDAQAPKIAAQHDKIQQAADKEILHLPNLTEEQRNKFRQSLRDDPSVSAEILAEAKKLNDAQAPKC

SEQ ID NO: 31 - protein, 365 aa, Artificial Sequence
  fusion protein 212897 (fusion of 212434 dimer with (PAdelFc)4)
AVLDIAQHSATEEIWWLPNLTKQQKVWFIMSLTQDPSVSKEVLGEAQKLNDSQAPKQAPKVDAKFDQAPKVDAKFDAVLDIAQHSATEEIWWLPNLTKQQKVWFIMSLTQDPSVSKEVLGEAQKLNDSQAPKIAAQHDKIQQAADKEILHLPNLTEEQRNKFRQSLRDDPSVSAEILAEAKKLNDAQAPKIAAQHDKIQQAADKEILHLPNLTEEQRNKFRQSLRDDPSVSAEILAEAKKLNDAQAPKIAAQHDKIQQAADKEILHLPNLTEEQRNKFRQSLRDDPSVSAEILAEAKKLNDAQAPKIAAQHDKIQQAADKEILHLPNLTEEQRNKFRQSLRDDPSVSAEILAEAKKLNDAQAPKC

SEQ ID NO: 32 - protein, 230 aa, Artificial Sequence
  fusion protein 213147  (213103 with (PAdelFc)2)
AKFDEAQQWAFYEILHLENLTEEQRNAFIQSLRDDPSVSREVLGEATKLNTSQAPKIAAKFDEAQLAAFQEIRHLPNLTEEQREAFITSLYDDPSVSLEVLGEAQKLNDSQAPKIAAQHDKIQQAADKEILHLPNLTEEQRNKFRQSLRDDPSVSAEILAEAKKLNDAQAPKIAAQHDKIQQAADKEILHLPNLTEEQRNKFRQSLRDDPSVSAEILAEAKKLNDAQAPK

SEQ ID NO: 33 - protein, 230 aa, Artificial Sequence
  fusion protein 213152 (212728 with (PAdelFc)2)
AKFDEAQLAAFEEIRHLPNLTEEQREAFITSLYDDPSVSLEVLGEAQKLNDSQAPKIAAKFDEAQQAAFYEILHLPNPTEWQRNYFIQQLRDDPSVSLAVLGRAQVLNDSQAPKIAAQHDKIQQAADKEILHLPNLTEEQRNKFRQSLRDDPSVSAEILAEAKKLNDAQAPKIAAQHDKIQQAADKEILHLPNLTEEQRNKFRQSLRDDPSVSAEILAEAKKLNDAQAPK

SEQ ID NO: 34 - protein, 114 aa, Artificial Sequence
  spike binding protein 213103 Ndel2
AKFDEAQQWAFYEILHLENLTEEQRNAFIQSLRDDPSVSREVLGEATKLNTSQAPKIAAKFDEAQLAAFQEIRHLPNLTEEQREAFITSLYDDPSVSLEVLGEAQKLNDSQAPK

SEQ ID NO: 35 - protein, 114 aa, Artificial Sequence
  spike binding protein 212728 Ndel2
AKFDEAQLAAFEEIRHLPNLTEEQREAFITSLYDDPSVSLEVLGEAQKLNDSQAPKIAAKFDEAQQAAFYEILHLPNPTEWQRNYFIQQLRDDPSVSLAVLGRAQVLNDSQAPK

SEQ ID NO: 36 - protein, 116 aa, Artificial Sequence
  spike binding protein 212880 (SEQ37+SEQ3)
IAAKFDEAQQLAFYLILHLINLTEEQRNAFIQSLRDDPSVSLEVLGEAYKLNLSQAPKIAAKFDEAQLAAFQEIRHLPNLTEEQREAFITSLYDDPSVSLEVLGEAQKLNDSQAPK

SEQ ID NO: 37 - protein, 58 aa, Artificial Sequence
  spike binding protein 212880 monomer
IAAKFDEAQQLAFYLILHLINLTEEQRNAFIQSLRDDPSVSLEVLGEAYKLNLSQAPK

SEQ ID NO: 38 - protein, 172 aa, Artificial Sequence
  fusion protein of SEQ28 with (PAdelFc)2
AVLDIDQHAATEEIWWLPNLTKQQKVWFIMSLTQDPSVSLEILAEAKKLNDAQAPKIAAQHDKIQQAADKEILHLPNLTEEQRNKFRQSLRDDPSVSAEILAEAKKLNDAQAPKIAAQHDKIQQAADKEILHLPNLTEEQRNKFRQSLRDDPSVSAEILAEAKKLNDAQAPK

SEQ ID NO: 39 - protein, 230 aa, Artificial Sequence
  fusion protein  of SEQ28-PAdelFc-SEQ28-PAdelFc
AVLDIDQHAATEEIWWLPNLTKQQKVWFIMSLTQDPSVSLEILAEAKKLNDAQAPKIAAQHDKIQQAADKEILHLPNLTEEQRNKFRQSLRDDPSVSAEILAEAKKLNDAQAPKIAAVLDIDQHAATEEIWWLPNLTKQQKVWFIMSLTQDPSVSLEILAEAKKLNDAQAPKIAAQHDKIQQAADKEILHLPNLTEEQRNKFRQSLRDDPSVSAEILAEAKKLNDAQAPK

SEQ ID NO: 40 - protein, 56 aa, Artificial Sequence
  spike protein binding protein
AKFDEAQQYAFYKILHLWNLTEEQRNAFIQSLRDDPSVSLEVLGEARKLNTSQAPK

SEQ ID NO: 41 - protein, 56 aa, Artificial Sequence
  spike binding protein 217800-1
AKFDEAQQYAFYKILHLWNLTEEQRNAFIQSLRDDPSVSLEILAEARKLNTAQAPK

SEQ ID NO: 42 - protein, 58 aa, Artificial Sequence
  spike protein binding protein 217800-2
IAAKFDEAQYAAFLEIVHLPNLTEEQRQAFIASLWDDPSVSLEILAEAKKLNDAQAPK

SEQ ID NO: 43 - protein, 114 aa, Artificial Sequence
  spike protein binding protein 217800
AKFDEAQQYAFYKILHLWNLTEEQRNAFIQSLRDDPSVSLEILAEARKLNTAQAPKIAAKFDEAQYAAFLEIVHLPNLTEEQRQAFIASLWDDPSVSLEILAEAKKLNDAQAPK

SEQ ID NO: 44 - protein, 114 aa, Artificial Sequence
  spike protein binding protein 217798
AKFDEAQQYAFYKILHLWNLTEEQRNAFIQSLRDDPSVSLEVLGEARKLNTSQAPKIAAKFDEAQYAAFLEIVHLPNLTEEQRQAFIASLWDDPSVSLEILAEAKKLNDAQAPK

SEQ ID NO: 45 - protein, 114 aa, Artificial Sequence
  spike protein binding protein (SEQ2 plus SEQ3)
AKFDEAQQYAFYKILHLWNLTEEQRNAFIQSLRDDPSVSLEVLGEARKLNTSQAPKIAAKFDEAQLAAFQEIRHLPNLTEEQREAFITSLYDDPSVSLEVLGEAQKLNDSQAPK

SEQ ID NO: 46 - protein, 230 aa, Artificial Sequence
  spike protein binding protein (217800 tetramer)
AKFDEAQQYAFYKILHLWNLTEEQRNAFIQSLRDDPSVSLEILAEARKLNTAQAPKIAAKFDEAQYAAFLEIVHLPNLTEEQRQAFIASLWDDPSVSLEILAEAKKLNDAQAPKIAAKFDEAQQYAFYKILHLWNLTEEQRNAFIQSLRDDPSVSLEILAEARKLNTAQAPKIAAKFDEAQYAAFLEIVHLPNLTEEQRQAFIASLWDDPSVSLEILAEAKKLNDAQAPK

SEQ ID NO: 47 - protein, 347 aa, Artificial Sequence
  212361 trimer (217797)
AKFDEAQQYAFYKILHLWNLTEEQRNAFIQSLRDDPSVSLEVLGEARKLNTSQAPKIAAKFDEAQYAAFLEIVHLPNLTEEQRQAFIASLWDDPSVSLEVLGEAQKLNDSQAPKIAAKFDEAQQYAFYKILHLWNLTEEQRNAFIQSLRDDPSVSLEVLGEARKLNTSQAPKIAAKFDEAQYAAFLEIVHLPNLTEEQRQAFIASLWDDPSVSLEVLGEAQKLNDSQAPKIAAKFDEAQQYAFYKILHLWNLTEEQRNAFIQSLRDDPSVSLEVLGEARKLNTSQAPKIAAKFDEAQYAAFLEIVHLPNLTEEQRQAFIASLWDDPSVSLEVLGEAQKLNDSQAPKC

SEQ ID NO: 48 - protein, 231 aa, Artificial Sequence
  Fusion protein 217238 (212361 fused to (PAdelFc)2)
AKFDEAQQYAFYKILHLWNLTEEQRNAFIQSLRDDPSVSLEVLGEARKLNTSQAPKIAAKFDEAQYAAFLEIVHLPNLTEEQRQAFIASLWDDPSVSLEVLGEAQKLNDSQAPKIAAQHDKIQQAADKEILHLPNLTEEQRNKFRQSLRDDPSVSAEILAEAKKLNDAQAPKIAAQHDKIQQAADKEILHLPNLTEEQRNKFRQSLRDDPSVSAEILAEAKKLNDAQAPKC

SEQ ID NO: 49 - protein, 231 aa, Artificial Sequence
  Fusion protein 218898
AKFDEAQQYAFYKILHLWNLTEEQRNAFIQSLRDDPSVSLEVLGEARKLNTSQAPKIAAKFDEAQYAAFLEIVHLPNLTEEQRQAFIASLWDDPSVSLEILAEAKKLNDAQAPKIAAQHDKIQQAADKEILHLPNLTEEQRNKFRQSLRDDPSVSAEILAEAKKLNDAQAPKIAAQHDKIQQAADKEILHLPNLTEEQRNKFRQSLRDDPSVSAEILAEAKKLNDAQAPKC

SEQ ID NO: 50 - protein, 347 aa, Artificial Sequence
  Fusion protein 217799
AKFDEAQQYAFYKILHLWNLTEEQRNAFIQSLRDDPSVSLEVLGEARKLNTSQAPKIAAKFDEAQYAAFLEIVHLPNLTEEQRQAFIASLWDDPSVSLEILAEAKKLNDAQAPKIAAKFDEAQQYAFYKILHLWNLTEEQRNAFIQSLRDDPSVSLEVLGEARKLNTSQAPKIAAKFDEAQYAAFLEIVHLPNLTEEQRQAFIASLWDDPSVSLEILAEAKKLNDAQAPKIAAQHDKIQQAADKEILHLPNLTEEQRNKFRQSLRDDPSVSAEILAEAKKLNDAQAPKIAAQHDKIQQAADKEILHLPNLTEEQRNKFRQSLRDDPSVSAEILAEAKKLNDAQAPKC

SEQ ID NO: 51 - protein, 231 aa, Artificial Sequence
  Fusion protein 217800
AKFDEAQQYAFYKILHLWNLTEEQRNAFIQSLRDDPSVSLEILAEARKLNTAQAPKIAAKFDEAQYAAFLEIVHLPNLTEEQRQAFIASLWDDPSVSLEILAEAKKLNDAQAPKIAAQHDKIQQAADKEILHLPNLTEEQRNKFRQSLRDDPSVSAEILAEAKKLNDAQAPKIAAQHDKIQQAADKEILHLPNLTEEQRNKFRQSLRDDPSVSAEILAEAKKLNDAQAPKC

SEQ ID NO: 52 - protein, 231 aa, Artificial Sequence
  Fusion protein SEQ28xSEQ43xPAdelFc
AVLDIDQHAATEEIWWLPNLTKQQKVWFIMSLTQDPSVSLEILAEAKKLNDAQAPKIAAKFDEAQQYAFYKILHLWNLTEEQRNAFIQSLRDDPSVSLEILAEARKLNTAQAPKIAAKFDEAQYAAFLEIVHLPNLTEEQRQAFIASLWDDPSVSLEILAEAKKLNDAQAPKIAAQHDKIQQAADKEILHLPNLTEEQRNKFRQSLRDDPSVSAEILAEAKKLNDAQAPKC

SEQ ID NO: 53 - protein, 231 aa, Artificial Sequence
  Fusion protein (SEQ43xSEQ28xPAdelFc)
AKFDEAQQYAFYKILHLWNLTEEQRNAFIQSLRDDPSVSLEILAEARKLNTAQAPKIAAKFDEAQYAAFLEIVHLPNLTEEQRQAFIASLWDDPSVSLEILAEAKKLNDAQAPKIAAVLDIDQHAATEEIWWLPNLTKQQKVWFIMSLTQDPSVSLEILAEAKKLNDAQAPKIAAQHDKIQQAADKEILHLPNLTEEQRNKFRQSLRDDPSVSAEILAEAKKLNDAQAPKC

SEQ ID NO: 54 - protein, 288 aa, Artificial Sequence
  Fusion protein (217800 dimer x PAdelFc)
AKFDEAQQYAFYKILHLWNLTEEQRNAFIQSLRDDPSVSLEILAEARKLNTAQAPKIAAKFDEAQYAAFLEIVHLPNLTEEQRQAFIASLWDDPSVSLEILAEAKKLNDAQAPKIAAKFDEAQQYAFYKILHLWNLTEEQRNAFIQSLRDDPSVSLEILAEARKLNTAQAPKIAAKFDEAQYAAFLEIVHLPNLTEEQRQAFIASLWDDPSVSLEILAEAKKLNDAQAPKIAAQHDKIQQAADKEILHLPNLTEEQRNKFRQSLRDDPSVSAEILAEAKKLNDAQAPK

SEQ ID NO: 55 - protein, 346 aa, Artificial Sequence
  Fusion protein 217800 x PAdelFc
AKFDEAQQYAFYKILHLWNLTEEQRNAFIQSLRDDPSVSLEILAEARKLNTAQAPKIAAKFDEAQYAAFLEIVHLPNLTEEQRQAFIASLWDDPSVSLEILAEAKKLNDAQAPKIAAKFDEAQQYAFYKILHLWNLTEEQRNAFIQSLRDDPSVSLEILAEARKLNTAQAPKIAAKFDEAQYAAFLEIVHLPNLTEEQRQAFIASLWDDPSVSLEILAEAKKLNDAQAPKIAAQHDKIQQAADKEILHLPNLTEEQRNKFRQSLRDDPSVSAEILAEAKKLNDAQAPKIAAQHDKIQQAADKEILHLPNLTEEQRNKFRQSLRDDPSVSAEILAEAKKLNDAQAPK

SEQ ID NO: 56 - protein, 229 aa, Artificial Sequence
  Fusion protein 217382 (212361 W20P) (no binding to spike protein)
AKFDEAQQYAFYKILHLPNLTEEQRNAFIQSLRDDPSVSLEVLGEARKLNTSQAPKIAAKFDEAQYAAFLEIVHLPNLTEEQRQAFIASLWDDPSVSLEVLGEAQKLNDSQAPKAQHDKIQQAADKEILHLPNLTEEQRNKFRQSLRDDPSVSAEILAEAKKLNDAQAPKIAAQHDKIQQAADKEILHLPNLTEEQRNKFRQSLRDDPSVSAEILAEAKKLNDAQAPKC

SEQ ID NO: 57 - protein, 114 aa, Artificial Sequence
  Spike binding protein 212864 (LQRETY-group)
AKFDEAQQQAFYRILHLINLTEEQRNAFIQSLRDDPSVSTEVLGEAQKLNTSQAPKIAAKFDEAQLAAFQEIRHLPNLTEEQREAFITSLYDDPSVSLEVLGEAQKLNDSQAPK

SEQ ID NO: 58 - protein, 114 aa, Artificial Sequence
  Spike protein binding protein 213102 (LQRETY-group)
AKFDEAQQAAFYLILHLHNLTEEQRNAFIQSLRDDPSVSYEVLGEAQKLNLSQAPKIAAKFDEAQLAAFQEIRHLPNLTEEQREAFITSLYDDPSVSLEVLGEAQKLNDSQAPK

SEQ ID NO: 59 - protein, 114 aa, Artificial Sequence
  spike protein binding protein 213101 (LQRETY-group)
AKFDEAQQQAFYHILHLWNLTEEQRNAFIQSLRDDPSVSTEVLGEAEKLNISQAPKIAAKFDEAQLAAFQEIRHLPNLTEEQREAFITSLYDDPSVSLEVLGEAQKLNDSQAPK

SEQ ID NO: 60 - protein, 114 aa, Artificial Sequence
  spike protein binding protein 212853 (LQRETY-group)
AKFDEAQQYAFYWILHLWNLTEEQRNAFIQSLRDDPSVSWEVLGEAYKLNLSQAPKIAAKFDEAQLAAFQEIRHLPNLTEEQREAFITSLYDDPSVSLEVLGEAQKLNDSQAPK

SEQ ID NO: 61 - protein, 114 aa, Artificial Sequence
  spike protein binding protein 213100 (LQRETY group)
AKFDEAQLAAFQEIRHLPNLTEEQREAFITSLYDDPSVSLEVLGEAQKLNDSQAPKIAAKFDEAQQAAFYEILHLPNLTEKQRNHFIQILRDDPSVSLRVLGYAQHLNDSQAPK

SEQ ID NO: 62 - protein, 114 aa, Artificial Sequence
  spike protein binding protein 213099 (LQRETY-group)
AKFDEAQLAAFQEIRHLPNLTEEQREAFITSLYDDPSVSLEVLGEAQKLNDSQAPKIAAKFDEAQQAAFYEILHLPNLTEHQRNAFIQWLRDDPSVSLQVLGHAQQLNDSQAPK

SEQ ID NO: 63 - protein, 114 aa, Artificial Sequence
  Spike protein binding protein SEQ28 dimer
AVLDIDQHAATEEIWWLPNLTKQQKVWFIMSLTQDPSVSLEILAEAKKLNDAQAPKIAAVLDIDQHAATEEIWWLPNLTKQQKVWFIMSLTQDPSVSLEILAEAKKLNDAQAPK

SEQ ID NO: 64 - protein, 114 aa, Artificial Sequence
  spike protein binding protein SEQ ID NO: 1dimer
AVLDIAQHSATEEIWWLPNLTKQQKVWFIMSLTQDPSVSKEVLGEAQKLNDSQAPKNAAVLDIAQHSATEEIWWLPNLTKQQKVWFIMSLTQDPSVSKEVLGEAQKLNDSQAPK

SEQ ID NO: 65 - protein, 58 aa, Artificial Sequence
  spike protein binding protein 434 consensus
  Xaa (8)..(8): Xaa may be selected from A or D
  Xaa (11)..(11): Xaa may be selected from S or A
  Xaa (42)..(42): Xaa may be selected from K or L
  Xaa (44)..(44): Xaa may be selected from V or I
  Xaa (46)..(46): Xaa may be selected from G or A
  Xaa (49)..(49): Xaa may be selected from Q or K
  Xaa (54)..(54): Xaa may be selected from S or A
NAAVLDIXQHXATEEIWWLPNLTKQQKVWFIMSLTQDPSVSXEXLXEAXKLNDXQAPK

SEQ ID NO: 66 - protein, 114 aa, Artificial Sequence
  Spike protein binding protein dimer 212361del2N
AKFDEAQQYAFYKILHLWNLTEEQRNAFIQSLRDDPSVSLEVLGEARKLNTSQAPKIAAKFDEAQYAAFLEIVHLPNLTEEQRQAFIASLWDDPSVSLEVLGEAQKLNDSQAPK

SEQ ID NO: 67 - protein, 114 aa, Artificial Sequence
  spike protein binding protein dimer 212335del2N
AKFDEAQQYAFYKILHLWNLTEEQRNAFIQSLRDDPSVSLEVLGEARKLNTSQAPKIAAKFDEAQYAAFLEIHHLPNLTEEQRHAFILSLYDDPSVSLEVLGEAQKLNDSQAPK

SEQ ID NO: 68 - protein, 347 aa, Artificial Sequence
  fusion protein of SEQ43 x (PAdelFc)3 x SEQ28
AKFDEAQQYAFYKILHLWNLTEEQRNAFIQSLRDDPSVSLEILAEARKLNTAQAPKIAAKFDEAQYAAFLEIVHLPNLTEEQRQAFIASLWDDPSVSLEILAEAKKLNDAQAPKIAAQHDKIQQAADKEILHLPNLTEEQRNKFRQSLRDDPSVSAEILAEAKKLNDAQAPKIAAQHDKIQQAADKEILHLPNLTEEQRNKFRQSLRDDPSVSAEILAEAKKLNDAQAPKIAAQHDKIQQAADKEILHLPNLTEEQRNKFRQSLRDDPSVSAEILAEAKKLNDAQAPKIAAVLDIDQHAATEEIWWLPNLTKQQKVWFIMSLTQDPSVSLEILAEAKKLNDAQAPKC

SEQ ID NO: 69 - protein, 289 aa, Artificial Sequence
  fusion protein of SEQ43 x (PAdelFc)2 x SEQ28
AKFDEAQQYAFYKILHLWNLTEEQRNAFIQSLRDDPSVSLEILAEARKLNTAQAPKIAAKFDEAQYAAFLEIVHLPNLTEEQRQAFIASLWDDPSVSLEILAEAKKLNDAQAPKIAAQHDKIQQAADKEILHLPNLTEEQRNKFRQSLRDDPSVSAEILAEAKKLNDAQAPKIAAQHDKIQQAADKEILHLPNLTEEQRNKFRQSLRDDPSVSAEILAEAKKLNDAQAPKIAAVLDIDQHAATEEIWWLPNLTKQQKVWFIMSLTQDPSVSLEILAEAKKLNDAQAPKC

SEQ ID NO: 70 - protein, 231 aa, Artificial Sequence
  fusion protein of SEQ43 x (PAdelFc)1 x SEQ28
AKFDEAQQYAFYKILHLWNLTEEQRNAFIQSLRDDPSVSLEILAEARKLNTAQAPKIAAKFDEAQYAAFLEIVHLPNLTEEQRQAFIASLWDDPSVSLEILAEAKKLNDAQAPKIAAQHDKIQQAADKEILHLPNLTEEQRNKFRQSLRDDPSVSAEILAEAKKLNDAQAPKIAAVLDIDQHAATEEIWWLPNLTKQQKVWFIMSLTQDPSVSLEILAEAKKLNDAQAPKC

SEQ ID NO: 71 - protein, 289 aa, Artificial Sequence
  fusion protein of SEQ28 x SEQ43 x (PAdelFc)2
AVLDIDQHAATEEIWWLPNLTKQQKVWFIMSLTQDPSVSLEILAEAKKLNDAQAPKIAAKFDEAQQYAFYKILHLWNLTEEQRNAFIQSLRDDPSVSLEILAEARKLNTAQAPKIAAKFDEAQYAAFLEIVHLPNLTEEQRQAFIASLWDDPSVSLEILAEAKKLNDAQAPKIAAQHDKIQQAADKEILHLPNLTEEQRNKFRQSLRDDPSVSAEILAEAKKLNDAQAPKIAAQHDKIQQAADKEILHLPNLTEEQRNKFRQSLRDDPSVSAEILAEAKKLNDAQAPKC

SEQ ID NO: 72 - protein, 289 aa, Artificial Sequence
  fusion protein of SEQ43 x SEQ28 x (PAdelFc)2
AKFDEAQQYAFYKILHLWNLTEEQRNAFIQSLRDDPSVSLEILAEARKLNTAQAPKIAAKFDEAQYAAFLEIVHLPNLTEEQRQAFIASLWDDPSVSLEILAEAKKLNDAQAPKIAAVLDIDQHAATEEIWWLPNLTKQQKVWFIMSLTQDPSVSLEILAEAKKLNDAQAPKIAAQHDKIQQAADKEILHLPNLTEEQRNKFRQSLRDDPSVSAEILAEAKKLNDAQAPKIAAQHDKIQQAADKEILHLPNLTEEQRNKFRQSLRDDPSVSAEILAEAKKLNDAQAPKC